European Patent Application EP 4 299 075 A1, published January 3, 2024. Title: COMBINATION THERAPY BASED ON PD-1 SIGNALING INHIBITORS. Applicant: Kyoto University. The sequence listing filed with the application follows.

SEQUENCE LISTING (10 sequences)

SEQ ID NO: 1 - DNA, 20 bp, Artificial Sequence
  primer
ccagagtgctgtggcaactc

SEQ ID NO: 2 - DNA, 20 bp, Artificial Sequence
  primer
gcaaacacaggctgttcctg

SEQ ID NO: 3 - DNA, 20 bp, Artificial Sequence
  primer
gacagttgaggacacctggc

SEQ ID NO: 4 - DNA, 20 bp, Artificial Sequence
  primer
ccagagaggagtgacatctc

SEQ ID NO: 5 - DNA, 21 bp, Artificial Sequence
  primer
tggcctcggcagaattggaag

SEQ ID NO: 6 - DNA, 22 bp, Artificial Sequence
  primer
tgtcattcagcaagcctgtggt

SEQ ID NO: 7 - DNA, 24 bp, Artificial Sequence
  primer
gatgaacatcccatttcgcattgg

SEQ ID NO: 8 - DNA, 24 bp, Artificial Sequence
  primer
gcgttatacagagaggcacgaatg

SEQ ID NO: 9 - DNA, 18 bp, Artificial Sequence
  primer
taaggccaaccgtgaaag

SEQ ID NO: 10 - DNA, 20 bp, Artificial Sequence
  primer
gaggcatacagggacagcac